European Patent Specification EP 3 294 321 B1, published July 31, 2024. Title: METHODS OF DETERMINING INTERFERON HAVING DIRECT INHIBITORY EFFECTS ON TUMORS AND USES THEREOF. Applicant: Superlab Far East Limited. The sequence listing filed with the application follows.

SEQUENCE LISTING (21 sequences)

SEQ ID NO: 1 - protein, 167 aa, Artificial Sequence
  Amino acid sequence of recombinant interferon
MCDLPQTHSLGNRRALILLAQMRRISPFSCLKDRHDFGFPQEEFDGNQFQKAQAISVLHEMIQQTFNLFSTKDSSAAWDESLLEKFYTELYQQLNDLEACVIQEVGVEETPLMNVDSILAVKKYFQRITLYLTEKKYSPCAWEVVRAEIMRSFSLSTNLQERLRRKE

SEQ ID NO: 2 - DNA, 504 bp, Artificial Sequence
  Nucleotide sequence encoding recombinant interferon
atgtgcgacctgccgcagacccactccctgggtaaccgtcgtgctctgatcctgctggctcagatgcgtcgtatctccccgttctcctgcctgaaagaccgtcacgacttcggtttcccgcaggaagaattcgacggtaaccagttccagaaagctcaggctatctccgttctgcacgaaatgatccagcagaccttcaacctgttctccaccaaagactcctccgctgcttgggacgaatccctgctggaaaaattctacaccgaactgtaccagcagctgaacgacctggaagcttgcgttatccaggaagttggtgttgaagaaaccccgctgatgaacgttgactccatcctggctgttaaaaaatacttccagcgtatcaccctgtacctgaccgaaaaaaaatactccccgtgcgcttgggaagttgttcgtgctgaaatcatgcgttccttctccctgtccaccaacctgcaggaacgtctgcgtcgtaaagaataa

SEQ ID NO: 3 - DNA, 504 bp, Artificial Sequence
  Nucleotide sequence encoding recombinant interferon
tacacgctggacggcgtctgggtgagggacccattggcagcacgagactaggacgaccgagtctacgcagcatagaggggcaagaggacggactttctggcagtgctgaagccaaagggcgtccttcttaagctgccattggtcaaggtctttcgagtccgatagaggcaagacgtgctttactaggtcgtctggaagttggacaagaggtggtttctgaggaggcgacgaaccctgcttagggacgacctttttaagatgtggcttgacatggtcgtcgacttgctggaccttcgaacgcaataggtccttcaaccacaacttctttggggcgactacttgcaactgaggtaggaccgacaattttttatgaaggtcgcatagtgggacatggactggcttttttttatgaggggcacgcgaacccttcaacaagcacgactttagtacgcaaggaagagggacaggtggttggacgtccttgcagacgcagcatttcttatt

SEQ ID NO: 4 - DNA, 20 bp, Artificial Sequence
  Sense primer
tgaagaaccagcaccacagg

SEQ ID NO: 5 - DNA, 22 bp, Artificial Sequence
  Antisense primer
cataaccaagaggcacagaagc

SEQ ID NO: 6 - DNA, 23 bp, Artificial Sequence
  Sense primer
gcggagtgaaggaaggattagtc

SEQ ID NO: 7 - DNA, 23 bp, Artificial Sequence
  Antisense primer
tgaacaagcagagatgtggaacc

SEQ ID NO: 8 - DNA, 18 bp, Artificial Sequence
  Sense primer
cgtggataccttagactt

SEQ ID NO: 9 - DNA, 18 bp, Artificial Sequence
  Antisense primer
gctgttgttctcaatgta

SEQ ID NO: 10 - DNA, 24 bp, Artificial Sequence
  Sense primer
tgaagaacatgtgagaggtttgac

SEQ ID NO: 11 - DNA, 24 bp, Artificial Sequence
  Antisense primer
gaaaactgaatctccattccacaa

SEQ ID NO: 12 - DNA, 20 bp, Artificial Sequence
  Sense primer
accgcatctctacattcaag

SEQ ID NO: 13 - DNA, 18 bp, Artificial Sequence
  Antisense primer
caagtctggctcgttctc

SEQ ID NO: 14 - DNA, 18 bp, Artificial Sequence
  Sense primer
cacaacaacaacaacaac

SEQ ID NO: 15 - DNA, 18 bp, Artificial Sequence
  Antisense primer
cacagtccaagtaagaga

SEQ ID NO: 16 - DNA, 20 bp, Artificial Sequence
  Sense primer
cagagcagggagcacaaacc

SEQ ID NO: 17 - DNA, 20 bp, Artificial Sequence
  Antisense primer
tgagcagaggagagcagagg

SEQ ID NO: 18 - DNA, 21 bp, Artificial Sequence
  Sense primer
ggagcctgactgaagagatgg

SEQ ID NO: 19 - DNA, 20 bp, Artificial Sequence
  Antisense primer
acgcctaaagcacacacctg

SEQ ID NO: 20 - DNA, 23 bp, Artificial Sequence
  Sense primer
ccttcaacctggcggacatcaac

SEQ ID NO: 21 - DNA, 18 bp, Artificial Sequence
  Antisense primer
ggctgctgcggcggaatg